European Patent Specification EP 3 574 115 B1, published July 26, 2023. Title: Nucleic Acid Detection Method. Applicant: Sense Biodetection Limited. The sequence listing filed with the application follows.

SEQUENCE LISTING (27 sequences)

SEQ ID NO: 1 - DNA, 40 bp, Artificial Sequence
  Oligonucleotide
atatatatataggagtctcggcatctatatatatatatat

SEQ ID NO: 2 - DNA, 43 bp, Artificial Sequence
  Oligonucleotide
atatatatatatatatttgagtcatagagatgccgagactcct

SEQ ID NO: 3 - DNA, 37 bp, Artificial Sequence
  Oligonucleotide
tttttttttttttttgagagccaggaccaggaacaca

SEQ ID NO: 4 - DNA, 37 bp, Artificial Sequence
  Oligonucleotide
ttttttttttttttttgtgttcctggtcctggctctc

SEQ ID NO: 5 - DNA, 25 bp, Artificial Sequence
  Oligonucleotide
attaataccatcaaaatgtatatat

SEQ ID NO: 6 - DNA, 21 bp, Artificial Sequence
  Oligonucleotide
atatatacattttgatggtat

SEQ ID NO: 7 - DNA, 21 bp, Artificial Sequence
  Oligonucleotide
atatatacattttgaaggtat

SEQ ID NO: 8 - DNA, 13 bp, Artificial Sequence
  Oligonucleotide
attttgatggtat

SEQ ID NO: 9 - DNA, 102 bp, Artificial Sequence
  Oligonucleotide
ttactgaggatattgcttgaagctggcagtgcctctcgatccgaatgctcagagacagaagagcgcaatggggactcttactgaggatattgcttgaagctg

SEQ ID NO: 10 - DNA, 42 bp, Artificial Sequence
  Oligonucleotide
aaaaaaaaaagtaaaagagtctgtccatcactaaaaaaaaaa

SEQ ID NO: 11 - DNA, 40 bp, Artificial Sequence
  Oligonucleotide
atatatatatattaaaccaagtaccgcactatatatatat

SEQ ID NO: 12 - DNA, 34 bp, Artificial Sequence
  Oligonucleotide
atatatatatcgcagtctctgaatatatatatat

SEQ ID NO: 13 - DNA, 38 bp, Artificial Sequence
  Oligonucleotide
aaaaaaaaaagagaggcactgccagcttaaaaaaaaaa

SEQ ID NO: 14 - DNA, 39 bp, Artificial Sequence
  Oligonucleotide
atatatatacgccagccattgcaacaggaatatatatat

SEQ ID NO: 15 - DNA, 44 bp, Artificial Sequence
  Oligonucleotide
atatatatatatattttcgtctcgattcgatatcttgactcctt

SEQ ID NO: 16 - DNA, 32 bp, Artificial Sequence
  Oligonucleotide
ttcttcttcttggtctcactcatgaggacgcc

SEQ ID NO: 17 - DNA, 32 bp, Artificial Sequence
  Oligonucleotide
ttcttcttcttggtctccaggagaccggtctt

SEQ ID NO: 18 - DNA, 36 bp, Artificial Sequence
  Oligonucleotide
caggagaccggtcttcccgagggcgtcctcaggagt

SEQ ID NO: 19 - DNA, 46 bp, Artificial Sequence
  Oligonucleotide
ccttgtgttcaccggtcttcccgagggtttttcttcttcttttttt

SEQ ID NO: 20 - DNA, 32 bp, Artificial Sequence; identical to SEQ ID NO: 16
  Oligonucleotide

SEQ ID NO: 21 - DNA, 32 bp, Artificial Sequence
  Oligonucleotide
ttgttgttgttggtctcggagaccggatcgtt

SEQ ID NO: 22 - DNA, 60 bp, Artificial Sequence
  Oligonucleotide
tgtccatgtttttttggagaccggatcgttacggcgtcctcatgagtaaaaatgtccatg

SEQ ID NO: 23 - DNA, 43 bp, Artificial Sequence
  Oligonucleotide
ccttgtgttcccggatcgttacggcttttcttcttcttttttt

SEQ ID NO: 24 - DNA, 33 bp, Artificial Sequence
  Oligonucleotide
gttgttgtgcttcccgaggacgccaatagagga

SEQ ID NO: 25 - DNA, 33 bp, Artificial Sequence
  Oligonucleotide
gttgttgtgcttcccgagtagaggcaggtgacc

SEQ ID NO: 26 - DNA, 64 bp, Artificial Sequence
  Oligonucleotide
tgtccatgttttttttagaggcaggtgaccggtctcctctattggcgtccaaaaaatgtccatg

SEQ ID NO: 27 - DNA, 43 bp, Artificial Sequence
  Oligonucleotide
ccttgtgttcccggtctcctctattgtttttcttcttcttttt